European Patent Specification EP 4 147 047 B1, published August 27, 2025. Title: Bioinformatics. Applicant: University of Helsinki. The sequence listing filed with the application follows.

SEQUENCE LISTING (80 sequences)

SEQ ID NO: 1 - protein, 9 aa, Artificial Sequence
  ELISspot peptide 1
SYHPALNAI

SEQ ID NO: 2 - protein, 9 aa, Artificial Sequence
  ELISpot peptide 2
SYLTSASSL

SEQ ID NO: 3 - protein, 9 aa, Artificial Sequence
  ELISpot peptide 3
YYVRILSTI

SEQ ID NO: 4 - protein, 9 aa, Artificial Sequence
  ELISpot peptide 4
SYLPPGTSL

SEQ ID NO: 5 - protein, 9 aa, Artificial Sequence
  ELISpot peptide 5
RYLPAPTAL

SEQ ID NO: 6 - protein, 9 aa, Artificial Sequence
  ELISpot peptide 6
KYIPAARHL

SEQ ID NO: 7 - protein, 9 aa, Artificial Sequence
  ELISpot peptide 7
AFHSSRTSL

SEQ ID NO: 8 - protein, 9 aa, Artificial Sequence
  ELISspot peptide 8
NYNSVNTRM

SEQ ID NO: 9 - protein, 9 aa, Artificial Sequence
  ELISpot peptide 9
SYSDMKRAL

SEQ ID NO: 10 - protein, 9 aa, Artificial Sequence
  ELISpot peptide 10
FYEKNKTLV

SEQ ID NO: 11 - protein, 9 aa, Artificial Sequence
  ELISpot peptide 11
KGPNRGVII

SEQ ID NO: 12 - protein, 9 aa, Artificial Sequence
  ELISpot peptide 12
FYKNGRLAV

SEQ ID NO: 13 - protein, 9 aa, Artificial Sequence
  ELISpot peptide 13
LYKESLSRL

SEQ ID NO: 14 - protein, 9 aa, Artificial Sequence
  ELISpot peptide 14
SYRDVIQEL

SEQ ID NO: 15 - protein, 9 aa, Artificial Sequence
  ELISspot peptide 15
KFYDSKETV

SEQ ID NO: 16 - protein, 9 aa, Artificial Sequence
  ELISpot peptide 16
KYLNVREAV

SEQ ID NO: 17 - protein, 9 aa, Artificial Sequence
  ELISspot peptide 17
HYLPDLHHM

SEQ ID NO: 18 - protein, 9 aa, Artificial Sequence
  ELISpot peptide 18
SGPNRFILI

SEQ ID NO: 19 - protein, 9 aa, Artificial Sequence
  ELISpot peptide 19
SYIIGTSSV

SEQ ID NO: 20 - protein, 9 aa, Artificial Sequence
  ELISpot peptide 20
RGPYVYREF

SEQ ID NO: 21 - protein, 9 aa, Artificial Sequence
  ELISpot peptide 21
FYATIIHDL

SEQ ID NO: 22 - protein, 9 aa, Artificial Sequence
  ELISpot peptide 22
GYMTPGLTV

SEQ ID NO: 23 - protein, 9 aa, Artificial Sequence
  ELISpot peptide 23
SYLIGRQKI

SEQ ID NO: 24 - protein, 9 aa, Artificial Sequence
  ELISpot peptide 24
AGASRIIGI

SEQ ID NO: 25 - protein, 8 aa, Artificial Sequence
  ELISspot peptide 25
QPEYIERL

SEQ ID NO: 26 - protein, 9 aa, Artificial Sequence
  ELISpot peptide 26
SYIHQRYIL

SEQ ID NO: 27 - protein, 9 aa, Artificial Sequence
  ELISspot peptide 27
SPSYAYHQF

SEQ ID NO: 28 - protein, 15 aa, Artificial Sequence
  polylysine peptide
KKKKKKSYLPPGTSL

SEQ ID NO: 29 - protein, 15 aa, Artificial Sequence
  polylysine peptide
KKKKKKRYLPAPTAL

SEQ ID NO: 30 - protein, 14 aa, Artificial Sequence
  polylysine polypeptide
KKKKKKYIPAARHL

SEQ ID NO: 31 - protein, 15 aa, Artificial Sequence
  polylysine peptide
KKKKKKLYKESLSRL

SEQ ID NO: 32 - protein, 15 aa, Artificial Sequence
  polylysine peptide
KKKKKKKYLNVREAV

SEQ ID NO: 33 - protein, 16 aa, Artificial Sequence
  polylysine peptide
KKKKKKKFYATIIHDL

SEQ ID NO: 34 - protein, 15 aa, Artificial Sequence
  polylysine peptide
KKKKKKSPSYAYHQF

SEQ ID NO: 35 - protein, 9 aa, Artificial Sequence
  Viral peptide herpesvirus 2
LPWHRLFLL

SEQ ID NO: 36 - protein, 9 aa, Artificial Sequence
  viral peptide pool 1 orthoreovirus
FAWPRLFEL

SEQ ID NO: 37 - protein, 9 aa, Artificial Sequence
  viral peptide pool 1 orthoreovirus
LRWTRLALL

SEQ ID NO: 38 - protein, 9 aa, Artificial Sequence
  viral peptide pool 1 strain ad169
LYGHRLFRL

SEQ ID NO: 39 - protein, 9 aa, Artificial Sequence
  viral peptide pool 1 lister
LFLHLLQLL

SEQ ID NO: 40 - protein, 9 aa, Artificial Sequence
  trp2
SVYDFFVWL

SEQ ID NO: 41 - protein, 9 aa, Artificial Sequence
  viral peptide pool 2 metapneumovirus
LNYDFFEAL

SEQ ID NO: 42 - protein, 9 aa, Artificial Sequence
  viral peptide pool 2 influenza
SVNSFFSRL

SEQ ID NO: 43 - protein, 9 aa, Artificial Sequence
  viral peptide pool 2 viral core cystein proteinase vaccinia
KVYTFFKFL

SEQ ID NO: 44 - protein, 9 aa, Artificial Sequence
  viral peptide pool 2 protein ul32 herpes
SNYSFFVQA

SEQ ID NO: 45 - protein, 9 aa, Artificial Sequence
  viral peptide pool 3
KVPRNQDWL

SEQ ID NO: 46 - protein, 9 aa, Artificial Sequence
  viral peptide pool 3 capsid protein papillomavirus
KVPLNADVL

SEQ ID NO: 47 - protein, 9 aa, Artificial Sequence
  viral peptide pool 3 orfla protein enteric coronavirus
KATRNNCWL

SEQ ID NO: 48 - protein, 9 aa, Artificial Sequence
  viral peptide pool 3 epstein barr virus
AVARNTDIL

SEQ ID NO: 49 - protein, 9 aa, Artificial Sequence
  viral peptide pool 3 echovirus
IVVRNHDDL

SEQ ID NO: 50 - protein, 9 aa, Homo sapiens
LLDTRTLEV

SEQ ID NO: 51 - protein, 9 aa, Homo sapiens
AMASASSSA

SEQ ID NO: 52 - protein, 9 aa, Homo sapiens
EILDVPSTV

SEQ ID NO: 53 - protein, 9 aa, Homo sapiens
MLARLASAA

SEQ ID NO: 54 - protein, 9 aa, Homo sapiens
NMMGLYDGM

SEQ ID NO: 55 - protein, 9 aa, Human cytomegalovirus
MLDRRTVEM

SEQ ID NO: 56 - protein, 9 aa, Human cytomegalovirus
AMAGASTSA

SEQ ID NO: 57 - protein, 9 aa, Human cytomegalovirus
DMMEMPATM

SEQ ID NO: 58 - protein, 9 aa, Human cytomegalovirus
FLTRLAEAA

SEQ ID NO: 59 - protein, 9 aa, Human cytomegalovirus
CMMTMYGGI

SEQ ID NO: 60 - protein, 9 aa, Molluscum contagiosum virus
SYHAALNAL

SEQ ID NO: 61 - protein, 9 aa, Human adenovirus type 31
HFSTSRTSL

SEQ ID NO: 62 - protein, 9 aa, Cercopithecine herpesvirus 1
AYQDTKRAL

SEQ ID NO: 63 - protein, 9 aa, Human herpesvirus 7
FYNSVNTRN

SEQ ID NO: 64 - protein, 9 aa, Influenza A virus
TIWTSASSI

SEQ ID NO: 65 - protein, 9 aa, epstein-barr virus
TYLPPSTSS

SEQ ID NO: 66 - protein, 9 aa, Orf virus
NYYKNKSLV

SEQ ID NO: 67 - protein, 9 aa, Human adenovirus type 41
AYMNGRVAV

SEQ ID NO: 68 - protein, 9 aa, Variola virus
KNPNRFVIF

SEQ ID NO: 69 - protein, 9 aa, Human cytomegalovirus
SHQPAARRL

SEQ ID NO: 70 - protein, 9 aa, Influenza C virus
RNMPAATAL

SEQ ID NO: 71 - protein, 9 aa, Human cytomegalovirus
SHQPAARRL

SEQ ID NO: 72 - protein, 9 aa, Molluscum contagiosum virus
YVFRLLSTI

SEQ ID NO: 73 - protein, 9 aa, Human cytomegalovirus
RYADVIQEV

SEQ ID NO: 74 - protein, 9 aa, Human adenovirus type 18
NFYNSKETV

SEQ ID NO: 75 - protein, 9 aa, Artificial Sequence
  MAGE A1 gene
KVLEYVIKV

SEQ ID NO: 76 - protein, 9 aa, Artificial Sequence
  HSP90 gene
ILDKKVEKV

SEQ ID NO: 77 - protein, 9 aa, Artificial Sequence
  PSME3
QLVDIIEKV

SEQ ID NO: 78 - protein, 10 aa, Artificial Sequence
  NNMT gene
VIMDALKSSY

SEQ ID NO: 79 - protein, 9 aa, Artificial Sequence
  FGA gene
FLAEGGGVR

SEQ ID NO: 80 - protein, 10 aa, Artificial Sequence
  HSPG2 gene
EVAQPGPSNR